European Patent Application EP 4 361 171 A2, published May 1, 2024. Title: ANTIBODY COMPOSITIONS FOR DISRUPTING BIOFILMS. Applicant: RESEARCH INSTITUTE AT NATIONWIDE CHILDREN'S HOSPITAL. Application EP. The sequence listing filed with the application follows.

SEQUENCE LISTING (99 sequences)

SEQ ID NO: 1 - protein, 473 aa, synthetic construct
  REGION 1..473: note = Description of Artificial Sequence: Synthetic polypeptide
MDPKGSLSWRILLFLSLAFELSYGEVKLVESGGGLVQPGGSLRLSCAASGFTFRTYAMSWVRQAPGKGLEWVATIGSDRRHTYYPDSVKGRFTISRDNAKNTLYLQMNSLRAEDTAVYYCVGPYDGYYGEFDYWGQGTLVTVSSASTKGPSVFPLAPSSKSTSGGTAALGCLVKDYFPEPVTVSWNSGALTSGVHTFPAVLQSSGLYSLSSVVTVPSSSLGTQTYICNVNHKPSNTKVDKKVEPKSCDKTHTCPPCPAPELLGGPSVFLFPPKPKDTLMISRTPEVTCVVVDVSHEDPEVKFNWYVDGVEVHNAKTKPREEQYNSTYRVVSVLTVLHQDWLNGKEYKCKVSNKALPAPIEKTISKAKGQPREPQVYTLPPSREEMTKNQVSLTCLVKGFYPSDIAVEWESNGQPENNYKTTPPVLDSDGSFFLYSKLTVDKSRWQQGNVFSCSVMHEALHNHYTQKSLSLSPG

SEQ ID NO: 2 - protein, 473 aa, synthetic construct
  REGION 1..473: note = Description of Artificial Sequence: Synthetic polypeptide
MDPKGSLSWRILLFLSLAFELSYGEVQLVESGGGLVQPGGSLRLSCAASGFTFRTYAMSWVRQAPGKGLEWVATIGSDRRHTYYPDSVKGRFTISRDNSKNTLYLQMNSLRAEDTAVYYCVGPYDGYYGEFDYWGQGTLVTVSSASTKGPSVFPLAPSSKSTSGGTAALGCLVKDYFPEPVTVSWNSGALTSGVHTFPAVLQSSGLYSLSSVVTVPSSSLGTQTYICNVNHKPSNTKVDKKVEPKSCDKTHTCPPCPAPELLGGPSVFLFPPKPKDTLMISRTPEVTCVVVDVSHEDPEVKFNWYVDGVEVHNAKTKPREEQYNSTYRVVSVLTVLHQDWLNGKEYKCKVSNKALPAPIEKTISKAKGQPREPQVYTLPPSREEMTKNQVSLTCLVKGFYPSDIAVEWESNGQPENNYKTTPPVLDSDGSFFLYSKLTVDKSRWQQGNVFSCSVMHEALHNHYTQKSLSLSPG

SEQ ID NO: 3 - protein, 473 aa, synthetic construct
  REGION 1..473: note = Description of Artificial Sequence: Synthetic polypeptide
MDPKGSLSWRILLFLSLAFELSYGEVKLVQSGAEVKKPGASVKVSCKASGFTFRTYAMSWVRQAPGQRLEWVATIGSDRRHTYYPDKFQGRVTITRDNAKNTLYMELSSLRSEDTAVYYCVGPYDGYYGEFDYWGQGTLVTVSSASTKGPSVFPLAPSSKSTSGGTAALGCLVKDYFPEPVTVSWNSGALTSGVHTFPAVLQSSGLYSLSSVVTVPSSSLGTQTYICNVNHKPSNTKVDKKVEPKSCDKTHTCPPCPAPELLGGPSVFLFPPKPKDTLMISRTPEVTCVVVDVSHEDPEVKFNWYVDGVEVHNAKTKPREEQYNSTYRVVSVLTVLHQDWLNGKEYKCKVSNKALPAPIEKTISKAKGQPREPQVYTLPPSREEMTKNQVSLTCLVKGFYPSDIAVEWESNGQPENNYKTTPPVLDSDGSFFLYSKLTVDKSRWQQGNVFSCSVMHEALHNHYTQKSLSLSPG

SEQ ID NO: 4 - protein, 473 aa, synthetic construct
  REGION 1..473: note = Description of Artificial Sequence: Synthetic polypeptide
MDPKGSLSWRILLFLSLAFELSYGEVQLVESGGGLVKPGGSLRLSCAASGFTFSRYGMSWVRQAPGKGLEWVATISSGGSYTYYTDSVKGRFTISRDNAKNSLYLQMNSLRAEDTAVYYCERHGGDGYWYFDVWGQGTMVTVSSASTKGPSVFPLAPSSKSTSGGTAALGCLVKDYFPEPVTVSWNSGALTSGVHTFPAVLQSSGLYSLSSVVTVPSSSLGTQTYICNVNHKPSNTKVDKKVEPKSCDKTHTCPPCPAPELLGGPSVFLFPPKPKDTLMISRTPEVTCVVVDVSHEDPEVKFNWYVDGVEVHNAKTKPREEQYNSTYRVVSVLTVLHQDWLNGKEYKCKVSNKALPAPIEKTISKAKGQPREPQVYTLPPSREEMTKNQVSLTCLVKGFYPSDIAVEWESNGQPENNYKTTPPVLDSDGSFFLYSKLTVDKSRWQQGNVFSCSVMHEALHNHYTQKSLSLSPG

SEQ ID NO: 5 - protein, 473 aa, synthetic construct
  REGION 1..473: note = Description of Artificial Sequence: Synthetic polypeptide
MDPKGSLSWRILLFLSLAFELSYGEVQLVESGGGLVKPGGSLRLSCAASGFTFSRYGMSWVRQAPGKGLEWVSTISSGGSYTYYTDSVKGRFTISRDNAKNSLYLQMNSLRAEDTAVYYCERHGGDGYWYFDVWGQGTMVTVSSASTKGPSVFPLAPSSKSTSGGTAALGCLVKDYFPEPVTVSWNSGALTSGVHTFPAVLQSSGLYSLSSVVTVPSSSLGTQTYICNVNHKPSNTKVDKKVEPKSCDKTHTCPPCPAPELLGGPSVFLFPPKPKDTLMISRTPEVTCVVVDVSHEDPEVKFNWYVDGVEVHNAKTKPREEQYNSTYRVVSVLTVLHQDWLNGKEYKCKVSNKALPAPIEKTISKAKGQPREPQVYTLPPSREEMTKNQVSLTCLVKGFYPSDIAVEWESNGQPENNYKTTPPVLDSDGSFFLYSKLTVDKSRWQQGNVFSCSVMHEALHNHYTQKSLSLSPG

SEQ ID NO: 6 - protein, 473 aa, synthetic construct
  REGION 1..473: note = Description of Artificial Sequence: Synthetic polypeptide
MDPKGSLSWRILLFLSLAFELSYGEVQLVESGGGLVQPGRSLRLSCTASGFTFSRYGMSWVRQAPGKGLEWVATISSGGSYTYYTDSVKGRFTISRDNAKNILYLQMNSLKTEDTAVYYCERHGGDGYWYFDVWGQGTMVTVSSASTKGPSVFPLAPSSKSTSGGTAALGCLVKDYFPEPVTVSWNSGALTSGVHTFPAVLQSSGLYSLSSVVTVPSSSLGTQTYICNVNHKPSNTKVDKKVEPKSCDKTHTCPPCPAPELLGGPSVFLFPPKPKDTLMISRTPEVTCVVVDVSHEDPEVKFNWYVDGVEVHNAKTKPREEQYNSTYRVVSVLTVLHQDWLNGKEYKCKVSNKALPAPIEKTISKAKGQPREPQVYTLPPSREEMTKNQVSLTCLVKGFYPSDIAVEWESNGQPENNYKTTPPVLDSDGSFFLYSKLTVDKSRWQQGNVFSCSVMHEALHNHYTQKSLSLSPG

SEQ ID NO: 7 - protein, 239 aa, synthetic construct
  REGION 1..239: note = Description of Artificial Sequence: Synthetic polypeptide
METDTLLLWVLLLWVPGSTGDVVMTQSPLSLPVTLGQPASISCRSSQSLLDSDGKTFLNWLQQRPGQSPRRLIYLVSKLDSGVPDRFSGSGSGTDFTLKISRVEAEDVGVYYCWQGTHFPYTFGQGTKLEIKRTVAAPSVFIFPPSDEQLKSGTASVVCLLNNFYPREAKVQWKVDNALQSGNSQESVTEQDSKDSTYSLSSTLTLSKADYEKHKVYACEVTHQGLSSPVTKSFNRGEC

SEQ ID NO: 8 - protein, 239 aa, synthetic construct
  REGION 1..239: note = Description of Artificial Sequence: Synthetic polypeptide
METDTLLLWVLLLWVPGSTGDVVMTQSPLSLPVTLGQPASISCRSSQSLLDSDGKTFLNWLQQRPGQSPRRLIYLVSKRDSGVPDRFSGSGSGTDFTLKISRVEAEDVGVYYCWQGTHFPYTFGQGTKLEIKRTVAAPSVFIFPPSDEQLKSGTASVVCLLNNFYPREAKVQWKVDNALQSGNSQESVTEQDSKDSTYSLSSTLTLSKADYEKHKVYACEVTHQGLSSPVTKSFNRGEC

SEQ ID NO: 9 - protein, 239 aa, synthetic construct
  REGION 1..239: note = Description of Artificial Sequence: Synthetic polypeptide
METDTLLLWVLLLWVPGSTGDVVMTQSPDSLAVSLGERATINCKSSQSLLDSDGKTFLNWLQQKPGQPPKRLIYLVSKLDSGVPDRFSGSGSGTDFTLTISSLQAEDVAVYYCWQGTHFPYTFGQGTKLEIKRTVAAPSVFIFPPSDEQLKSGTASVVCLLNNFYPREAKVQWKVDNALQSGNSQESVTEQDSKDSTYSLSSTLTLSKADYEKHKVYACEVTHQGLSSPVTKSFNRGEC

SEQ ID NO: 10 - protein, 233 aa, synthetic construct
  REGION 1..233: note = Description of Artificial Sequence: Synthetic polypeptide
METDTLLLWVLLLWVPGSTGDIQMTQSPSSLSASVGDRVTITCRASQDISNYLNWYQQKPGKAVKLLIYYTSRLHSGVPSRFSGSGSGTDYTLTISSLQPEDFATYFCQQGNPLRTFGGGTKVEIKRTVAAPSVFIFPPSDEQLKSGTASVVCLLNNFYPREAKVQWKVDNALQSGNSQESVTEQDSKDSTYSLSSTLTLSKADYEKHKVYACEVTHQGLSSPVTKSFNRGEC

SEQ ID NO: 11 - protein, 233 aa, synthetic construct
  REGION 1..233: note = Description of Artificial Sequence: Synthetic polypeptide
METDTLLLWVLLLWVPGSTGDIQMTQSPSSLSASVGDRVTITCRASQDISNYLNWYQQKPGKAVKLLIYYTSRLHSGVPSRFSGSGSGTDYTLTISSLQPEDFATYYCQQGNPLRTFGGGTKVEIKRTVAAPSVFIFPPSDEQLKSGTASVVCLLNNFYPREAKVQWKVDNALQSGNSQESVTEQDSKDSTYSLSSTLTLSKADYEKHKVYACEVTHQGLSSPVTKSFNRGEC

SEQ ID NO: 12 - protein, 233 aa, synthetic construct
  REGION 1..233: note = Description of Artificial Sequence: Synthetic polypeptide
METDTLLLWVLLLWVPGSTGDIVMTQSPATLSLSPGERATLSCRASQDISNYLNWYQQKPGQAVRLLIYYTSRLHSGIPARFSGSGSGTDYTLTISSLEPEDFAVYFCQQGNPLRTFGGGTKVEIKRTVAAPSVFIFPPSDEQLKSGTASVVCLLNNFYPREAKVQWKVDNALQSGNSQESVTEQDSKDSTYSLSSTLTLSKADYEKHKVYACEVTHQGLSSPVTKSFNRGEC

SEQ ID NO: 13 - protein, 473 aa, synthetic construct
  REGION 1..473: note = Description of Artificial Sequence: Synthetic polypeptide
  MOD_RES 27: note = Any amino acid, such as Q or K
  MOD_RES 30: note = Any amino acid, such as E or Q
  MOD_RES 33: note = Any amino acid, such as G or A
  MOD_RES 34: note = Any amino acid, such as G or E
  MOD_RES 35: note = Any amino acid, such as L or V
  MOD_RES 36: note = Any amino acid, such as V or K
  MOD_RES 37: note = Any amino acid, such as Q or K, or absent
  MOD_RES 40: note = Any amino acid, such as R, G or A
  MOD_RES 42: note = Any amino acid, such as L or V
  MOD_RES 43: note = Any amino acid, such as R or K
  MOD_RES 44: note = Any amino acid, such as L or V
  MOD_RES 47: note = Any amino acid, such as T, A or K
  MOD_RES 54: note = Any amino acid, such as S or R, or absent
  MOD_RES 55: note = Any amino acid, such as R or T, or absent
  MOD_RES 57: note = Any amino acid, such as G or A, or absent
  MOD_RES 67: note = Any amino acid, such as K or Q
  MOD_RES 68: note = Any amino acid, such as G or R
  MOD_RES 73: note = Any amino acid, such as A or S
  MOD_RES 76: note = Any amino acid, such as S or G, or absent
  MOD_RES 78: note = Any amino acid, such as G or D, or absent
  MOD_RES 79: note = Any amino acid, such as G or R, or absent
  MOD_RES 80: note = Any amino acid, such as S or R, or absent
  MOD_RES 81: note = Any amino acid, such as Y or H, or absent
  MOD_RES 85: note = Any amino acid, such as T or P, or absent
  MOD_RES 87: note = Any amino acid, such as S or K
  MOD_RES 88: note = Any amino acid, such as V or F
  MOD_RES 89: note = Any amino acid, such as K or Q
  MOD_RES 92: note = Any amino acid, such as F or V
  MOD_RES 95: note = Any amino acid, such as S or T
  MOD_RES 99: note = Any amino acid, such as A or S
  MOD_RES 102: note = Any amino acid, such as I, S or T
  MOD_RES 105: note = Any amino acid, such as L or M
  MOD_RES 106: note = Any amino acid, such as Q or E
  MOD_RES 107: note = Any amino acid, such as M or L
  MOD_RES 108: note = Any amino acid, such as N or S
  MOD_RES 111: note = Any amino acid, such as K or R
  MOD_RES 112: note = Any amino acid, such as T, A or S
  MOD_RES 121: note = Any amino acid, such as E or V, or absent
  MOD_RES 122: note = Any amino acid, such as R or G, or absent
  MOD_RES 123: note = Any amino acid, such as H or P, or absent
  MOD_RES 124: note = Any amino acid, such as G or Y, or absent
  MOD_RES 125: note = Any amino acid, such as G or D, or absent
  MOD_RES 126: note = Any amino acid, such as D or G, or absent
  MOD_RES 127: note = Any amino acid, such as G or Y, or absent
  MOD_RES 129: note = Any amino acid, such as W or G, or absent
  MOD_RES 130: note = Any amino acid, such as Y or E, or absent
  MOD_RES 133: note = Any amino acid, such as V or Y, or absent
  MOD_RES 139: note = Any amino acid, such as M or L, or absent
MDPKGSLSWRILLFLSLAFELSYGEVXLVXSGXXXXXPGXSXXXSCXASGFTFXXYXMSWVRQAPGXXLEWVXTIXSXXXXTYYXDXXXGRXTIXRDNXKNXLYXXXXSLXXEDTAVYYCXXXXXXXYXXFDXWGQGTXVTVSSASTKGPSVFPLAPSSKSTSGGTAALGCLVKDYFPEPVTVSWNSGALTSGVHTFPAVLQSSGLYSLSSVVTVPSSSLGTQTYICNVNHKPSNTKVDKKVEPKSCDKTHTCPPCPAPELLGGPSVFLFPPKPKDTLMISRTPEVTCVVVDVSHEDPEVKFNWYVDGVEVHNAKTKPREEQYNSTYRVVSVLTVLHQDWLNGKEYKCKVSNKALPAPIEKTISKAKGQPREPQVYTLPPSREEMTKNQVSLTCLVKGFYPSDIAVEWESNGQPENNYKTTPPVLDSDGSFFLYSKLTVDKSRWQQGNVFSCSVMHEALHNHYTQKSLSLSPG

SEQ ID NO: 14 - protein, 239 aa, synthetic construct
  REGION 1..239: note = Description of Artificial Sequence: Synthetic polypeptide
  MOD_RES 22: note = Any amino acid, such as I or V, or absent
  MOD_RES 23: note = Any amino acid, such as V or Q
  MOD_RES 29: note = Any amino acid, such as A, S, D or L, or absent
  MOD_RES 30: note = Any amino acid, such as T or S
  MOD_RES 32: note = Any amino acid, such as S, A or P
  MOD_RES 33: note = Any amino acid, such as L, A or V
  MOD_RES 34: note = Any amino acid, such as S or T
  MOD_RES 35: note = Any amino acid, such as P, V or L
  MOD_RES 37: note = Any amino acid, such as E, D or Q, or absent
  MOD_RES 38: note = Any amino acid, such as R or P
  MOD_RES 39: note = Any amino acid, such as A or V
  MOD_RES 40: note = Any amino acid, such as T or S
  MOD_RES 41: note = Any amino acid, such as L or I
  MOD_RES 42: note = Any amino acid, such as S, T or N
  MOD_RES 44: note = Any amino acid, such as R or K
  MOD_RES 45: note = Any amino acid, such as A or S, or absent
  MOD_RES 48: note = Any amino acid, such as D or S, or absent
  MOD_RES 49: note = Any amino acid, such as I or L, or absent
  MOD_RES 50: note = Any amino acid, such as L or absent
  MOD_RES 51: note = Any amino acid, such as D or absent
  MOD_RES 52: note = Any amino acid, such as S or absent
  MOD_RES 53: note = Any amino acid, such as D or absent
  MOD_RES 54: note = Any amino acid, such as G or absent
  MOD_RES 55: note = Any amino acid, such as S or K, or absent
  MOD_RES 56: note = Any amino acid, such as N or T, or absent
  MOD_RES 57: note = Any amino acid, such as Y or F, or absent
  MOD_RES 61: note = Any amino acid, such as Y or L, or absent
  MOD_RES 64: note = Any amino acid, such as K or R
  MOD_RES 67: note = Any amino acid, such as Q or K
  MOD_RES 68: note = Any amino acid, such as A, P or S
  MOD_RES 69: note = Any amino acid, such as V or P, or absent
  MOD_RES 70: note = Any amino acid, such as R or K, or absent
  MOD_RES 71: note = Any amino acid, such as L or R, or absent
  MOD_RES 75: note = Any amino acid, such as Y or L, or absent
  MOD_RES 76: note = Any amino acid, such as T or V, or absent
  MOD_RES 78: note = Any amino acid, such as R or K, or absent
  MOD_RES 79: note = Any amino acid, such as L or R
  MOD_RES 80: note = Any amino acid, such as H or D, or absent
  MOD_RES 83: note = Any amino acid, such as I or V
  MOD_RES 85: note = Any amino acid, such as A, S or D
  MOD_RES 96: note = Any amino acid, such as Y or F, or absent
  MOD_RES 99: note = Any amino acid, such as T or K
  MOD_RES 102: note = Any amino acid, such as S or R
  MOD_RES 103: note = Any amino acid, such as L or V
  MOD_RES 104: note = Any amino acid, such as E or Q, or absent
  MOD_RES 105: note = Any amino acid, such as P or A, or absent
  MOD_RES 108: note = Any amino acid, such as F or V, or absent
  MOD_RES 109: note = Any amino acid, such as A or G
  MOD_RES 110: note = Any amino acid, such as V or T
  MOD_RES 112: note = Any amino acid, such as F or Y
  MOD_RES 114: note = Any amino acid, such as Q or W, or absent
  MOD_RES 117: note = Any amino acid, such as N or T, or absent
  MOD_RES 118: note = Any amino acid, such as P or H, or absent
  MOD_RES 119: note = Any amino acid, such as F or absent
  MOD_RES 120: note = Any amino acid, such as L or P, or absent
  MOD_RES 121: note = Any amino acid, such as R or Y, or absent
  MOD_RES 125: note = Any amino acid, such as G or Q, or absent
  MOD_RES 129: note = Any amino acid, such as V or L, or absent
METDTLLLWVLLLWVPGSTGDXXMTQSPXXLXXXXGXXXXXXCXXSQXXXXXXXXXXLNWXQQXPGXXXXXLIYXXSXXXSGXPXRFSGSGSGTDXTLXISXXXXEDXXXYXCXQGXXXXXTFGXGTKXEIKRTVAAPSVFIFPPSDEQLKSGTASVVCLLNNFYPREAKVQWKVDNALQSGNSQESVTEQDSKDSTYSLSSTLTLSKADYEKHKVYACEVTHQGLSSPVTKSFNRGEC

SEQ ID NO: 15 - protein, 384 aa, Homo sapiens
APTKAPDVFPIISGCRHPKDNSPVVLACLITGYHPTSVTVTWYMGTQSQPQRTFPEIQRRDSYYMTSSQLSTPLQQWRQGEYKCVVQHTASKSKKEIFRWPESPKAQASSVPTAQPQAEGSLAKATTAPATTRNTGRGGEEKKKEKEKEEQEERETKTPECPSHTQPLGVYLLTPAVQDLWLRDKATFTCFVVGSDLKDAHLTWEVAGKVPTGGVEEGLLERHSNGSQSQHSRLTLPRSLWNAGTSVTCTLNHPSLPPQRLMALREPAAQAPVKLSLNLLASSDPPEAASWLLCEVSGFSPPNILLMWLEDQREVNTSGFAPARPPPQPGSTTFWAWSVLRVPAPPSPQPATYTCVVSHEDSRTLLNASRSLEVSYVTDHGPMK

SEQ ID NO: 16 - protein, 330 aa, Homo sapiens [sequence omitted]

SEQ ID NO: 17 - protein, 326 aa, Homo sapiens
ASTKGPSVFPLAPCSRSTSESTAALGCLVKDYFPEPVTVSWNSGALTSGVHTFPAVLQSSGLYSLSSVVTVPSSNFGTQTYTCNVDHKPSNTKVDKTVERKCCVECPPCPAPPVAGPSVFLFPPKPKDTLMISRTPEVTCVVVDVSHEDPEVQFNWYVDGVEVHNAKTKPREEQFNSTFRVVSVLTVVHQDWLNGKEYKCKVSNKGLPAPIEKTISKTKGQPREPQVYTLPPSREEMTKNQVSLTCLVKGFYPSDISVEWESNGQPENNYKTTPPMLDSDGSFFLYSKLTVDKSRWQQGNVFSCSVMHEALHNHYTQKSLSLSPGK

SEQ ID NO: 18 - protein, 377 aa, Homo sapiens
ASTKGPSVFPLAPCSRSTSGGTAALGCLVKDYFPEPVTVSWNSGALTSGVHTFPAVLQSSGLYSLSSVVTVPSSSLGTQTYTCNVNHKPSNTKVDKRVELKTPLGDTTHTCPRCPEPKSCDTPPPCPRCPEPKSCDTPPPCPRCPEPKSCDTPPPCPRCPAPELLGGPSVFLFPPKPKDTLMISRTPEVTCVVVDVSHEDPEVQFKWYVDGVEVHNAKTKPREEQYNSTFRVVSVLTVLHQDWLNGKEYKCKVSNKALPAPIEKTISKTKGQPREPQVYTLPPSREEMTKNQVSLTCLVKGFYPSDIAVEWESSGQPENNYNTTPPMLDSDGSFFLYSKLTVDKSRWQQGNIFSCSVMHEALHNRFTQKSLSLSPGK

SEQ ID NO: 19 - protein, 452 aa, Homo sapiens
GSASAPTLFPLVSCENSPSDTSSVAVGCLAQDFLPDSITLSWKYKNNSDISSTRGFPSVLRGGKYAATSQVLLPSKDVMQGTDEHVVCKVQHPNGNKEKNVPLPVIAELPPKVSVFVPPRDGFFGNPRKSKLICQATGFSPRQIQVSWLREGKQVGSGVTTDQVQAEAKESGPTTYKVTSTLTIKESDWLGQSMFTCRVDHRGLTFQQNASSMCVPDQDTAIRVFAIPPSFASIFLTKSTKLTCLVTDLTTYDSVTISWTRQNGEAVKTHTNISESHPNATFSAVGEASICEDDWNSGERFTCTVTHTDLPSPLKQTISRPKGVALHRPDVYLLPPAREQLNLRESATITCLVTGFSPADVFVQWMQRGQPLSPEKYVTSAPMPEPQAPGRYFAHSILTVSEEEWNTGETYTCVAHEALPNRVTERTVDKSTGKPTLYNVSLVMSDTAGTCY

SEQ ID NO: 20 - protein, 327 aa, Homo sapiens
ASTKGPSVFPLAPCSRSTSESTAALGCLVKDYFPEPVTVSWNSGALTSGVHTFPAVLQSSGLYSLSSVVTVPSSSLGTKTYTCNVDHKPSNTKVDKRVESKYGPPCPSCPAPEFLGGPSVFLFPPKPKDTLMISRTPEVTCVVVDVSQEDPEVQFNWYVDGVEVHNAKTKPREEQFNSTYRVVSVLTVLHQDWLNGKEYKCKVSNKGLPSSIEKTISKAKGQPREPQVYTLPPSQEEMTKNQVSLTCLVKGFYPSDIAVEWESNGQPENNYKTTPPVLDSDGSFFLYSRLTVDKSRWQEGNVFSCSVMHEALHNHYTQKSLSLSLGK

SEQ ID NO: 21 - protein, 353 aa, Homo sapiens
ASPTSPKVFPLSLCSTQPDGNVVIACLVQGFFPQEPLSVTWSESGQGVTARNFPPSQDASGDLYTTSSQLTLPATQCLAGKSVTCHVKHYTNPSQDVTVPCPVPSTPPTPSPSTPPTPSPSCCHPRLSLHRPALEDLLLGSEANLTCTLTGLRDASGVTFTWTPSSGKSAVQGPPERDLCGCYSVSSVLPGCAEPWNHGKTFTCTAAYPESKTPLTATLSKSGNTFRPEVHLLPPPSEELALNELVTLTCLARGFSPKDVLVRWLQGSQELPREKYLTWASRQEPSQGTTTFAVTSILRVAAEDWKKGDTFSCMVGHEALPLAFTQKTIDRLAGKPTHVNVSVVMAEVDGTCY

SEQ ID NO: 22 - protein, 340 aa, Homo sapiens
ASPTSPKVFPLSLDSTPQDGNVVVACLVQGFFPQEPLSVTWSESGQNVTARNFPPSQDASGDLYTTSSQLTLPATQCPDGKSVTCHVKHYTNPSQDVTVPCPVPPPPPCCHPRLSLHRPALEDLLLGSEANLTCTLTGLRDASGATFTWTPSSGKSAVQGPPERDLCGCYSVSSVLPGCAQPWNHGETFTCTAAHPELKTPLTANITKSGNTFRPEVHLLPPPSEELALNELVTLTCLARGFSPKDVLVRWLQGSQELPREKYLTWASRQEPSQGTTTFAVTSILRVAAEDWKKGDTFSCMVGHEALPLAFTQKTIDRMAGKPTHVNVSVVMAEVDGTCY

SEQ ID NO: 23 - protein, 106 aa, Homo sapiens
TVAAPSVFIFPPSDEQLKSGTASVVCLLNNFYPREAKVQWKVDNALQSGNSQESVTEQDSKDSTYSLSSTLTLSKADYEKHKVYACEVTHQGLSSPVTKSFNRGEC

SEQ ID NO: 24 - protein, 473 aa, synthetic construct
  REGION 1..473: note = Description of Artificial Sequence: Synthetic polypeptide
  MOD_RES 27: note = K or Q
  MOD_RES 30: note = Q or E
  MOD_RES 33: note = A or G
  MOD_RES 34: note = E or G
  MOD_RES 35: note = V or L
  MOD_RES 36: note = K or V
  MOD_RES 37: note = K or Q
  MOD_RES 40: note = A or G
  MOD_RES 42: note = V or L
  MOD_RES 43: note = K or R
  MOD_RES 44: note = V or L
  MOD_RES 47: note = K or A
  MOD_RES 67: note = Q or K
  MOD_RES 68: note = R or G
  MOD_RES 87: note = K or S
  MOD_RES 88: note = F or V
  MOD_RES 89: note = Q or K
  MOD_RES 92: note = V or F
  MOD_RES 95: note = T or S
  MOD_RES 99: note = A or S
  MOD_RES 105: note = M or L
  MOD_RES 106: note = E or Q
  MOD_RES 107: note = L or M
  MOD_RES 108: note = S or N
  MOD_RES 112: note = S or A
MDPKGSLSWRILLFLSLAFELSYGEVXLVXSGXXXXXPGXSXXXSCXASGFTFRTYAMSWVRQAPGXXLEWVATIGSDRRHTYYPDXXXGRXTIXRDNXKNTLYXXXXSLRXEDTAVYYCVGPYDGYYGEFDYWGQGTLVTVSSASTKGPSVFPLAPSSKSTSGGTAALGCLVKDYFPEPVTVSWNSGALTSGVHTFPAVLQSSGLYSLSSVVTVPSSSLGTQTYICNVNHKPSNTKVDKKVEPKSCDKTHTCPPCPAPELLGGPSVFLFPPKPKDTLMISRTPEVTCVVVDVSHEDPEVKFNWYVDGVEVHNAKTKPREEQYNSTYRVVSVLTVLHQDWLNGKEYKCKVSNKALPAPIEKTISKAKGQPREPQVYTLPPSREEMTKNQVSLTCLVKGFYPSDIAVEWESNGQPENNYKTTPPVLDSDGSFFLYSKLTVDKSRWQQGNVFSCSVMHEALHNHYTQKSLSLSPG

SEQ ID NO: 25 - protein, 239 aa, synthetic construct
  REGION 1..239: note = Description of Artificial Sequence: Synthetic polypeptide
  MOD_RES 29: note = D or L
  MOD_RES 32: note = A or P
  MOD_RES 34: note = S or T
  MOD_RES 37: note = E or Q
  MOD_RES 38: note = R or P
  MOD_RES 40: note = T or S
  MOD_RES 42: note = N or S
  MOD_RES 44: note = K or R
  MOD_RES 64: note = K or R
  MOD_RES 68: note = P or S
  MOD_RES 70: note = K or R
  MOD_RES 79: note = L or R
  MOD_RES 99: note = T or K
  MOD_RES 102: note = S or R
  MOD_RES 103: note = L or V
  MOD_RES 104: note = Q or E
  MOD_RES 109: note = A or G
METDTLLLWVLLLWVPGSTGDVVMTQSPXSLXVXLGXXAXIXCXSSQSLLDSDGKTFLNWLQQXPGQXPXRLIYLVSKXDSGVPDRFSGSGSGTDFTLXISXXXAEDVXVYYCWQGTHFPYTFGQGTKLEIKRTVAAPSVFIFPPSDEQLKSGTASVVCLLNNFYPREAKVQWKVDNALQSGNSQESVTEQDSKDSTYSLSSTLTLSKADYEKHKVYACEVTHQGLSSPVTKSFNRGEC

SEQ ID NO: 26 - protein, 473 aa, synthetic construct
  REGION 1..473: note = Description of Artificial Sequence: Synthetic polypeptide
  MOD_RES 37: note = Q or K
  MOD_RES 40: note = R or G
  MOD_RES 47: note = T or A
  MOD_RES 73: note = A or S
  MOD_RES 102: note = I or S
  MOD_RES 111: note = K or R
  MOD_RES 112: note = T or A
MDPKGSLSWRILLFLSLAFELSYGEVQLVESGGGLVXPGXSLRLSCXASGFTFSRYGMSWVRQAPGKGLEWVXTISSGGSYTYYTDSVKGRFTISRDNAKNXLYLQMNSLXXEDTAVYYCERHGGDGYWYFDVWGQGTMVTVSSASTKGPSVFPLAPSSKSTSGGTAALGCLVKDYFPEPVTVSWNSGALTSGVHTFPAVLQSSGLYSLSSVVTVPSSSLGTQTYICNVNHKPSNTKVDKKVEPKSCDKTHTCPPCPAPELLGGPSVFLFPPKPKDTLMISRTPEVTCVVVDVSHEDPEVKFNWYVDGVEVHNAKTKPREEQYNSTYRVVSVLTVLHQDWLNGKEYKCKVSNKALPAPIEKTISKAKGQPREPQVYTLPPSREEMTKNQVSLTCLVKGFYPSDIAVEWESNGQPENNYKTTPPVLDSDGSFFLYSKLTVDKSRWQQGNVFSCSVMHEALHNHYTQKSLSLSPG

SEQ ID NO: 27 - protein, 233 aa, synthetic construct
  REGION 1..233: note = Description of Artificial Sequence: Synthetic polypeptide
  MOD_RES 23: note = V or Q
  MOD_RES 29: note = A or S
  MOD_RES 30: note = T or S
  MOD_RES 33: note = L or A
  MOD_RES 35: note = P or V
  MOD_RES 37: note = E or D
  MOD_RES 39: note = A or V
  MOD_RES 41: note = L or I
  MOD_RES 42: note = S or T
  MOD_RES 62: note = Q or K
  MOD_RES 65: note = R or K
  MOD_RES 78: note = I or V
  MOD_RES 80: note = A or S
  MOD_RES 99: note = E or Q
  MOD_RES 105: note = V or T
  MOD_RES 107: note = F or Y
METDTLLLWVLLLWVPGSTGDIXMTQSPXXLSXSXGXRXTXXCRASQDISNYLNWYQQKPGXAVXLLIYYTSRLHSGXPXRFSGSGSGTDYTLTISSLXPEDFAXYXCQQGNPLRTFGGGTKVEIKRTVAAPSVFIFPPSDEQLKSGTASVVCLLNNFYPREAKVQWKVDNALQSGNSQESVTEQDSKDSTYSLSSTLTLSKADYEKHKVYACEVTHQGLSSPVTKSFNRGEC

SEQ ID NO: 28 - skipped

SEQ ID NO: 29 - protein, 90 aa, Escherichia coli
MNKTQLIDVIAEKAELSKTQAKAALESTLAAITESLKEGDAVQLVGFGTFKVNHRAERTGRNPQTGKEIKIAAANVPAFVSGKALKDAVK

SEQ ID NO: 30 - protein, 90 aa, Escherichia coli
MNKSQLIDKIAAGADISKAAAGRALDAIIASVTESLKEGDDVALVGFGTFAVKERAARTGRNPQTGKEITIAAAKVPSFRAGKALKDAVN

SEQ ID NO: 31 - protein, 21 aa, Haemophilus influenzae
NFELRDKSSRPGRNPKTGDVV

SEQ ID NO: 32 - protein, 21 aa, Haemophilus influenzae
SLHHRQPRLGRNPKTGDSVNL

SEQ ID NO: 33 - protein, 6 aa, synthetic construct
  REGION 1..6: note = Description of Artificial Sequence: Synthetic peptide
GPSLKL

SEQ ID NO: 34 - protein, 4 aa, synthetic construct
  REGION 1..4: note = Description of Artificial Sequence: Synthetic peptide
GPSL

SEQ ID NO: 35 - protein, 4 aa, synthetic construct
  REGION 1..4: note = Description of Artificial Sequence: Synthetic peptide
PSLK

SEQ ID NO: 36 - protein, 5 aa, synthetic construct
  REGION 1..5: note = Description of Artificial Sequence: Synthetic peptide
GPSLK

SEQ ID NO: 37 - protein, 4 aa, synthetic construct
  REGION 1..4: note = Description of Artificial Sequence: Synthetic peptide
SLKL

SEQ ID NO: 38 - protein, 60 aa, synthetic construct
  REGION 1..60: note = Description of Artificial Sequence: Synthetic polypeptide
  MOD_RES 7: note = Any amino acid
  MOD_RES 21..40: note = Any amino acid
  SITE 21..40: note = This region may encompass 1-20 residues
  MOD_RES 55: note = Any amino acid
RPGRNPXTGDVVPVSARRVVXXXXXXXXXXXXXXXXXXXXFSLHHRQPRLGRNPXTGDSV

SEQ ID NO: 39 - protein, 60 aa, synthetic construct
  REGION 1..60: note = Description of Artificial Sequence: Synthetic polypeptide
  MOD_RES 21..40: note = Any amino acid
  SITE 21..40: note = This region may encompass 1-20 residues
RPGRNPKTGDVVPVSARRVVXXXXXXXXXXXXXXXXXXXXFSLHHRQPRLGRNPKTGDSV

SEQ ID NO: 40 - protein, 44 aa, synthetic construct
  REGION 1..44: note = Description of Artificial Sequence: Synthetic polypeptide
RPGRNPKTGDVVPVSARRVVGPSLFSLHHRQPRLGRNPKTGDSV

SEQ ID NO: 41 - protein, 60 aa, synthetic construct
  REGION 1..60: note = Description of Artificial Sequence: Synthetic polypeptide
  MOD_RES 21..40: note = Any amino acid
  SITE 21..40: note = This region may encompass 1-20 residues
FLEEIRLSLESGQDVKLSGFXXXXXXXXXXXXXXXXXXXXTLSAKEIENMVKDILEFISQ

SEQ ID NO: 42 - protein, 6 aa, synthetic construct
  REGION 1..6: note = Description of Artificial Sequence: Synthetic peptide
GGSGGS

SEQ ID NO: 43 - protein, 6 aa, synthetic construct
  REGION 1..6: note = Description of Artificial Sequence: Synthetic peptide
GPSLKL

SEQ ID NO: 44 - skipped

SEQ ID NO: 45 - protein, 4 aa, synthetic construct
  REGION 1..4: note = Description of Artificial Sequence: Synthetic peptide
GPSL

SEQ ID NO: 46 - skipped

SEQ ID NO: 47 - protein, 4 aa, synthetic construct
  REGION 1..4: note = Description of Artificial Sequence: Synthetic peptide
PSLK

SEQ ID NO: 48 - protein, 5 aa, synthetic construct
  REGION 1..5: note = Description of Artificial Sequence: Synthetic peptide
GPSLK

SEQ ID NO: 49 - protein, 4 aa, synthetic construct
  REGION 1..4: note = Description of Artificial Sequence: Synthetic peptide
SLKL

SEQ ID NO: 50 - protein, 44 aa, synthetic construct
  REGION 1..44: note = Description of Artificial Sequence: Synthetic polypeptide
FLEEIRLSLESGQDVKLSGFGPSLTLSAKEIENMVKDILEFISQ

SEQ ID NO: 51 - protein, 7 aa, synthetic construct
  REGION 1..7: note = Description of Artificial Sequence: Synthetic peptide
  MOD_RES 5: note = Any amino acid, such as S or R
  MOD_RES 6: note = Any amino acid, such as R or T
GFTFXXY

SEQ ID NO: 52 - protein, 7 aa, synthetic construct
  REGION 1..7: note = Description of Artificial Sequence: Synthetic peptide
GFTFRTY

SEQ ID NO: 53 - protein, 6 aa, synthetic construct
  REGION 1..6: note = Description of Artificial Sequence: Synthetic peptide
GSDRRH

SEQ ID NO: 54 - protein, 13 aa, synthetic construct
  REGION 1..13: note = Description of Artificial Sequence: Synthetic peptide
VGPYDGYYGEFDY

SEQ ID NO: 55 - protein, 7 aa, synthetic construct
  REGION 1..7: note = Description of Artificial Sequence: Synthetic peptide
GFTFSRY

SEQ ID NO: 56 - protein, 6 aa, synthetic construct
  REGION 1..6: note = Description of Artificial Sequence: Synthetic peptide
SSGGSY

SEQ ID NO: 57 - protein, 13 aa, synthetic construct
  REGION 1..13: note = Description of Artificial Sequence: Synthetic peptide
ERHGGDGYWYFDV

SEQ ID NO: 58 - protein, 11 aa, synthetic construct
  REGION 1..11: note = Description of Artificial Sequence: Synthetic peptide
QSLLDSDGKTF

SEQ ID NO: 59 - protein, 7 aa, synthetic construct
  REGION 1..7: note = Description of Artificial Sequence: Synthetic peptide
WQGTHFP

SEQ ID NO: 60 - protein, 8 aa, synthetic construct
  REGION 1..8: note = Description of Artificial Sequence: Synthetic peptide
GFTFRTYA

SEQ ID NO: 61 - protein, 13 aa, synthetic construct
  REGION 1..13: note = Description of Artificial Sequence: Synthetic peptide
  MOD_RES 1: note = A or K
XASGFTFRTYAMS

SEQ ID NO: 62 - protein, 8 aa, synthetic construct
  REGION 1..8: note = Description of Artificial Sequence: Synthetic peptide
IGSDRRHT

SEQ ID NO: 63 - protein, 9 aa, synthetic construct
  REGION 1..9: note = Description of Artificial Sequence: Synthetic peptide
IGSDRRHTY

SEQ ID NO: 64 - protein, 10 aa, synthetic construct
  REGION 1..10: note = Description of Artificial Sequence: Synthetic peptide
TIGSDRRHTY

SEQ ID NO: 65 - protein, 15 aa, synthetic construct
  REGION 1..15: note = Description of Artificial Sequence: Synthetic peptide
WVATIGSDRRHTYYP

SEQ ID NO: 66 - protein, 16 aa, synthetic construct
  REGION 1..16: note = Description of Artificial Sequence: Synthetic peptide
  MOD_RES 1: note = R or K
XSSQSLLDSDGKTFLN

SEQ ID NO: 67 - protein, 7 aa, synthetic construct
  REGION 1..7: note = Description of Artificial Sequence: Synthetic peptide
  MOD_RES 5: note = L or R
LVSKXDS

SEQ ID NO: 68 - protein, 8 aa, synthetic construct
  REGION 1..8: note = Description of Artificial Sequence: Synthetic peptide
  MOD_RES 6: note = L or R
YLVSKXDS

SEQ ID NO: 69 - protein, 8 aa, synthetic construct
  REGION 1..8: note = Description of Artificial Sequence: Synthetic peptide
  MOD_RES 5: note = L or R
LVSKXDSG

SEQ ID NO: 70 - protein, 10 aa, synthetic construct
  REGION 1..10: note = Description of Artificial Sequence: Synthetic peptide
  MOD_RES 6: note = L or R
YLVSKXDSGV

SEQ ID NO: 71 - protein, 15 aa, synthetic construct
  REGION 1..15: note = Description of Artificial Sequence: Synthetic peptide
  MOD_RES 9: note = L or R
RLIYLVSKXDSGVPD

SEQ ID NO: 72 - protein, 8 aa, synthetic construct
  REGION 1..8: note = Description of Artificial Sequence: Synthetic peptide
WQGTHFPY

SEQ ID NO: 73 - protein, 9 aa, synthetic construct
  REGION 1..9: note = Description of Artificial Sequence: Synthetic peptide
WQGTHFPYT

SEQ ID NO: 74 - protein, 8 aa, synthetic construct
  REGION 1..8: note = Description of Artificial Sequence: Synthetic peptide
QQGNPLRT

SEQ ID NO: 75 - protein, 6 aa, synthetic construct
  REGION 1..6: note = Description of Artificial Sequence: Synthetic peptide
QDISNY

SEQ ID NO: 76 - protein, 8 aa, synthetic construct
  REGION 1..8: note = Description of Artificial Sequence: Synthetic peptide
YLVSKRDS

SEQ ID NO: 77 - protein, 16 aa, synthetic construct
  REGION 1..16: note = Description of Artificial Sequence: Synthetic peptide
KSSQSLLDSDGKTFLN

SEQ ID NO: 78 - protein, 13 aa, synthetic construct
  REGION 1..13: note = Description of Artificial Sequence: Synthetic peptide
KASGFTFRTYAMS

SEQ ID NO: 79 - protein, 7 aa, synthetic construct
  REGION 1..7: note = Description of Artificial Sequence: Synthetic peptide
LVSKRDS

SEQ ID NO: 80 - protein, 8 aa, synthetic construct
  REGION 1..8: note = Description of Artificial Sequence: Synthetic peptide
GFTFSRYG

SEQ ID NO: 81 - protein, 13 aa, synthetic construct
  REGION 1..13: note = Description of Artificial Sequence: Synthetic peptide
  MOD_RES 1: note = A or T
XASGFTFSRYGMS

SEQ ID NO: 82 - protein, 8 aa, synthetic construct
  REGION 1..8: note = Description of Artificial Sequence: Synthetic peptide
ISSGGSYT

SEQ ID NO: 83 - protein, 10 aa, synthetic construct
  REGION 1..10: note = Description of Artificial Sequence: Synthetic peptide
TISSGGSYTY

SEQ ID NO: 84 - protein, 11 aa, synthetic construct
  REGION 1..11: note = Description of Artificial Sequence: Synthetic peptide
RASQDISNYLN

SEQ ID NO: 85 - protein, 7 aa, synthetic construct
  REGION 1..7: note = Description of Artificial Sequence: Synthetic peptide
YTSRLHS

SEQ ID NO: 86 - protein, 8 aa, synthetic construct
  REGION 1..8: note = Description of Artificial Sequence: Synthetic peptide
YYTSRLHS

SEQ ID NO: 87 - protein, 13 aa, synthetic construct
  REGION 1..13: note = Description of Artificial Sequence: Synthetic peptide
TASGFTFSRYGMS

SEQ ID NO: 88 - protein, 120 aa, synthetic construct
  REGION 1..120: note = Description of Artificial Sequence: Synthetic polypeptide
EVQLVESGGGLVKPGGSLRLSCAASGFTFSRYGMSWVRQAPGKGLEWVATISSGGSYTYYTDSVKGRFTISRDNAKNSLYLQMNSLRAEDTAVYYCERHGGDGYWYFDVWGQGTMVTVSS

SEQ ID NO: 89 - protein, 120 aa, synthetic construct
  REGION 1..120: note = Description of Artificial Sequence: Synthetic polypeptide
EVQLVESGGGLVKPGGSLRLSCAASGFTFSRYGMSWVRQAPGKGLEWVSTISSGGSYTYYTDSVKGRFTISRDNAKNSLYLQMNSLRAEDTAVYYCERHGGDGYWYFDVWGQGTMVTVSS

SEQ ID NO: 90 - protein, 120 aa, synthetic construct
  REGION 1..120: note = Description of Artificial Sequence: Synthetic polypeptide
EVQLVESGGGLVQPGRSLRLSCTASGFTFSRYGMSWVRQAPGKGLEWVATISSGGSYTYYTDSVKGRFTISRDNAKNILYLQMNSLKTEDTAVYYCERHGGDGYWYFDVWGQGTMVTVSS

SEQ ID NO: 91 - protein, 106 aa, synthetic construct
  REGION 1..106: note = Description of Artificial Sequence: Synthetic polypeptide
DIQMTQSPSSLSASVGDRVTITCRASQDISNYLNWYQQKPGKAVKLLIYYTSRLHSGVPSRFSGSGSGTDYTLTISSLQPEDFATYFCQQGNPLRTFGGGTKVEIK

SEQ ID NO: 92 - protein, 106 aa, synthetic construct
  REGION 1..106: note = Description of Artificial Sequence: Synthetic polypeptide
DIQMTQSPSSLSASVGDRVTITCRASQDISNYLNWYQQKPGKAVKLLIYYTSRLHSGVPSRFSGSGSGTDYTLTISSLQPEDFATYYCQQGNPLRTFGGGTKVEIK

SEQ ID NO: 93 - protein, 106 aa, synthetic construct
  REGION 1..106: note = Description of Artificial Sequence: Synthetic polypeptide
DIVMTQSPATLSLSPGERATLSCRASQDISNYLNWYQQKPGQAVRLLIYYTSRLHSGIPARFSGSGSGTDYTLTISSLEPEDFAVYFCQQGNPLRTFGGGTKVEIK

SEQ ID NO: 94 - protein, 120 aa, synthetic construct
  REGION 1..120: note = Description of Artificial Sequence: Synthetic polypeptide
EVKLVESGGGLVQPGGSLRLSCAASGFTFRTYAMSWVRQAPGKGLEWVATIGSDRRHTYYPDSVKGRFTISRDNAKNTLYLQMNSLRAEDTAVYYCVGPYDGYYGEFDYWGQGTLVTVSS

SEQ ID NO: 95 - protein, 120 aa, synthetic construct
  REGION 1..120: note = Description of Artificial Sequence: Synthetic polypeptide
EVQLVESGGGLVQPGGSLRLSCAASGFTFRTYAMSWVRQAPGKGLEWVATIGSDRRHTYYPDSVKGRFTISRDNSKNTLYLQMNSLRAEDTAVYYCVGPYDGYYGEFDYWGQGTLVTVSS

SEQ ID NO: 96 - protein, 120 aa, synthetic construct
  REGION 1..120: note = Description of Artificial Sequence: Synthetic polypeptide
EVKLVQSGAEVKKPGASVKVSCKASGFTFRTYAMSWVRQAPGQRLEWVATIGSDRRHTYYPDKFQGRVTITRDNAKNTLYMELSSLRSEDTAVYYCVGPYDGYYGEFDYWGQGTLVTVSS

SEQ ID NO: 97 - protein, 112 aa, synthetic construct
  REGION 1..112: note = Description of Artificial Sequence: Synthetic polypeptide
DVVMTQSPLSLPVTLGQPASISCRSSQSLLDSDGKTFLNWLQQRPGQSPRRLIYLVSKLDSGVPDRFSGSGSGTDFTLKISRVEAEDVGVYYCWQGTHFPYTFGQGTKLEIK

SEQ ID NO: 98 - protein, 112 aa, synthetic construct
  REGION 1..112: note = Description of Artificial Sequence: Synthetic polypeptide
DVVMTQSPLSLPVTLGQPASISCRSSQSLLDSDGKTFLNWLQQRPGQSPRRLIYLVSKRDSGVPDRFSGSGSGTDFTLKISRVEAEDVGVYYCWQGTHFPYTFGQGTKLEIK

SEQ ID NO: 99 - protein, 112 aa, synthetic construct
  REGION 1..112: note = Description of Artificial Sequence: Synthetic polypeptide
DVVMTQSPDSLAVSLGERATINCKSSQSLLDSDGKTFLNWLQQKPGQPPKRLIYLVSKLDSGVPDRFSGSGSGTDFTLTISSLQAEDVAVYYCWQGTHFPYTFGQGTKLEIK